European Patent Specification EP 3 892 295 B1, published April 26, 2023. Title: INDIVIDUALIZED VACCINES FOR CANCER. Applicant: BioNTech RNA Pharmaceuticals GmbH et al. The sequence listing filed with the application follows.

SEQUENCE LISTING (39 sequences)

SEQ ID NO: 1 - protein, 15 aa, Artificial Sequence
  Linker sequence
  REPEAT (1)..(3): Portion of sequence repeated a times, wherein a is independently a number selected from 0, 1, 2, 3, 4, 5, 6, 7, 8, 9, 10, 11, 12, 13, 14, 15, 16, 17, 18, 19, or 20
  REPEAT (4)..(6): Portion of sequence repeated b times, wherein b is independently a number selected from 0, 1, 2, 3, 4, 5, 6, 7, 8, 9, 10, 11, 12, 13, 14, 15, 16, 17, 18, 19, or 20
  REPEAT (7)..(9): Portion of sequence repeated c times, wherein c is independently a number selected from 0, 1, 2, 3, 4, 5, 6, 7, 8, 9, 10, 11, 12, 13, 14, 15, 16, 17, 18, 19, or 20
  REPEAT (10)..(12): Portion of sequence repeated d times, wherein d is independently a number selected from 0, 1, 2, 3, 4, 5, 6, 7, 8, 9, 10, 11, 12, 13, 14, 15, 16, 17, 18, 19, or 20
  REPEAT (13)..(15): Portion of sequence repeated e times, wherein e is independently a number selected from 0, 1, 2, 3, 4, 5, 6, 7, 8, 9, 10, 11, 12, 13, 14, 15, 16, 17, 18, 19, or 20
  MISC_FEATURE (1)..(15): a + b + c + d + e are different from 0 and preferably are 2 or more, 3 or more, 4 or more or 5 or more
GGSGSSGGGSSGGSG

SEQ ID NO: 2 - protein, 9 aa, Artificial Sequence
  Linker sequence
GGSGGGGSG

SEQ ID NO: 3 - protein, 8 aa, Artificial Sequence
  Epitope sequence
SIINFEKL

SEQ ID NO: 4 - protein, 30 aa, Artificial Sequence
  Mutated peptide sequence
SPSKPSFQEFVDWENVSPELNSTDQPFLPS

SEQ ID NO: 5 - protein, 30 aa, Artificial Sequence
  Wildtype peptide sequence
SPSKPSFQEFVDWEKVSPELNSTDQPFLPS

SEQ ID NO: 6 - protein, 27 aa, Artificial Sequence
  Mutated peptide sequence
TPPPEEAMPFEFNGPAQGDHSQPPLQV

SEQ ID NO: 7 - protein, 27 aa, Artificial Sequence
  Wildtype peptide sequence
TPPPEEAMPFEFNEPAQGDHSQPPLQV

SEQ ID NO: 8 - protein, 27 aa, Artificial Sequence
  Mutated peptide sequence
RVTCNRAGEKHCFSSNEAARDFGGAIQ

SEQ ID NO: 9 - protein, 27 aa, Wildtype peptide sequence
RVTCNRAGEKHCFTSNEAARDFGGAIQ

SEQ ID NO: 10 - protein, 27 aa, Artificial Sequence
  Mutated peptide sequence
FRRKAFLHWYTGEAMDEMEFTEAESNM

SEQ ID NO: 11 - protein, 27 aa, Artificial Sequence
  Wildtype peptide sequence
FRRKAFLHWYTGEGMDEMEFTEAESNM

SEQ ID NO: 12 - protein, 27 aa, Artificial Sequence
  Mutated peptide sequence
PSKPSFQEFVDWENVSPELNSTDQPFL

SEQ ID NO: 13 - protein, 27 aa, Artificial Sequence
  Wildtype peptide sequence
PSKPSFQEFVDWEKVSPELNSTDQPFL

SEQ ID NO: 14 - protein, 27 aa, Artificial Sequence
  Mutated peptide sequence
HLTQQLDTYILKNVVAFSRTDKYRQLP

SEQ ID NO: 15 - protein, 27 aa, Artificial Sequence
  Wildtype peptide sequence
HLTQQLDTYILKNFVAFSRTDKYRQLP

SEQ ID NO: 16 - protein, 27 aa, Artificial Sequence
  Mutated peptide sequence
CGTAFFINFIAIYHHASRAIPFGTMVA

SEQ ID NO: 17 - protein, 27 aa, Artificial Sequence
  Wildtype peptide sequence
CGTAFFINFIAIYYHASRAIPFGTMVA

SEQ ID NO: 18 - protein, 7 aa, Artificial Sequence
  Linker sequence
GGSGGGG

SEQ ID NO: 19 - protein, 10 aa, Artificial Sequence
  Linker sequence
TSLNALLNAH

SEQ ID NO: 20 - protein, 10 aa, Artificial Sequence
  Linker sequence
SSSSSSSSSS

SEQ ID NO: 21 - protein, 10 aa, Artificial Sequence
  Linker sequence
GGGGGGGGGG

SEQ ID NO: 22 - protein, 10 aa, Artificial Sequence
  Linker sequence
GGSGGGGSGG

SEQ ID NO: 23 - protein, 10 aa, Artificial Sequence
  Linker sequence
GGSGGGSGGG

SEQ ID NO: 24 - protein, 9 aa, Artificial Sequence
  Linker sequence
TSLNALLNA

SEQ ID NO: 25 - protein, 9 aa, Artificial Sequence
  Linker sequence
SSSSSSSSS

SEQ ID NO: 26 - protein, 9 aa, Artificial Sequence
  Linker sequence
GGGGGGGGG

SEQ ID NO: 27 - protein, 9 aa, Artificial Sequence
  Linker sequence
GGSGGGSGG

SEQ ID NO: 28 - protein, 5 aa, Artificial Sequence
  Linker sequence
GGSGG

SEQ ID NO: 29 - protein, 6 aa, Artificial Sequence
  Linker sequence
GGSGGG

SEQ ID NO: 30 - protein, 7 aa, Artificial Sequence
  Linker sequence
GGSGGGG

SEQ ID NO: 31 - protein, 8 aa, Artificial Sequence
  Linker sequence
GGSGGGGS

SEQ ID NO: 32 - protein, 10 aa, Artificial Sequence
  Linker sequence
GGSGGGSGGS

SEQ ID NO: 33 - DNA, 14 bp, Artificial Sequence
  Oligonucleotide
ggaaactttttccc

SEQ ID NO: 34 - DNA, 21 bp, Artificial Sequence
  Oligonucleotide
ccggggaaactttttcccagt

SEQ ID NO: 35 - DNA, 21 bp, Artificial Sequence
  Oligonucleotide
ccggggaaacgttttcccagt

SEQ ID NO: 36 - protein, 60 aa, Artificial Sequence
  Artificial construct
NTTFNVSEESPSKPSFQEFVDWENVSPELNSTDQPFLPSAPVFIFTKGRKGGSGGGGSGG

SEQ ID NO: 37 - protein, 60 aa, Artificial Sequence
  Artificial construct
YFVLYKPPPKDNIPALVEEYLERGNFVANDLDWLLALPHDKFWCQVIFDEGGSGGGSGGS

SEQ ID NO: 38 - protein, 60 aa, Artificial Sequence
  Artificial construct
FEQLSESAKEELINFKRKRVAAFQKNLIEMSELEIKHARNNVSLLQSCIDGGSGGGGSGG

SEQ ID NO: 39 - protein, 60 aa, Artificial Sequence
  Artificial construct
TGASPGLGAYTPPPEEAMPFEFNGPAQGDHSQPPLQVPDLAPGGPEALVPGGSGGGSGGS